European Patent Application EP 4 574 169 A1, published June 25, 2025. Title: Pharmacetical Compositions comprising Herpes Simplex Virus Vectors. Applicant: Tomoki TODO. Application JP. The sequence listing filed with the application follows.

SEQUENCE LISTING (7 sequences)

SEQ ID NO: 1 - protein, 1273 aa, synthetic construct
MFVFLVLLPLVSSQCVNLTTRTQLPPAYTNSFTRGVYYPDKVFRSSVLHSTQDLFLPFFSNVTWFHAIHVSGTNGTKRFDNPVLPFNDGVYFASTEKSNIIRGWIFGTTLDSKTQSLLIVNNATNVVIKVCEFQFCNDPFLGVYYHKNNKSWMESEFRVYSSANNCTFEYVSQPFLMDLEGKQGNFKNLREFVFKNIDGYFKIYSKHTPINLVRDLPQGFSALEPLVDLPIGINITRFQTLLALHRSYLTPGDSSSGWTAGAAAYYVGYLQPRTFLLKYNENGTITDAVDCALDPLSETKCTLKSFTVEKGIYQTSNFRVQPTESIVRFPNITNLCPFGEVFNATRFASVYAWNRKRISNCVADYSVLYNSASFSTFKCYGVSPTKLNDLCFTNVYADSFVIRGDEVRQIAPGQTGKIADYNYKLPDDFTGCVIAWNSNNLDSKVGGNYNYLYRLFRKSNLKPFERDISTEIYQAGSTPCNGVEGFNCYFPLQSYGFQPTNGVGYQPYRVVVLSFELLHAPATVCGPKKSTNLVKNKCVNFNFNGLTGTGVLTESNKKFLPFQQFGRDIADTTDAVRDPQTLEILDITPCSFGGVSVITPGTNTSNQVAVLYQDVNCTEVPVAIHADQLTPTWRVYSTGSNVFQTRAGCLIGAEHVNNSYECDIPIGAGICASYQTQTNSPRRARSVASQSIIAYTMSLGAENSVAYSNNSIAIPTNFTISVTTEILPVSMTKTSVDCTMYICGDSTECSNLLLQYGSFCTQLNRALTGIAVEQDKNTQEVFAQVKQIYKTPPIKDFGGFNFSQILPDPSKPSKRSFIEDLLFNKVTLADAGFIKQYGDCLGDIAARDLICAQKFNGLTVLPPLLTDEMIAQYTSALLAGTITSGWTFGAGAALQIPFAMQMAYRFNGIGVTQNVLYENQKLIANQFNSAIGKIQDSLSSTASALGKLQDVVNQNAQALNTLVKQLSSNFGAISSVLNDILSRLDPPEAEVQIDRLITGRLQSLQTYVTQQLIRAAEIRASANLAATKMSECVLGQSKRVDFCGKGYHLMSFPQSAPHGVVFLHVTYVPAQEKNFTTAPAICHDGKAHFPREGVFVSNGTHWFVTQRNFYEPQIITTDNTFVSGNCDVVIGIVNNTVYDPLQPELDSFKEELDKYFKNHTSPDVDLGDISGINASVVNIQKEIDRLNEVAKNLNESLIDLQELGKYEQYIKWPWYIWLGFIAGLIAIVMVTIMLCCMTSCCSCLKGCCSCGSCCKFDEDDSEPVLKGVKLHYT

SEQ ID NO: 2 - protein, 1273 aa, synthetic construct
MFVFLVLLPLVSSQCVNLTTRTQLPPAYTNSFTRGVYYPDKVFRSSVLHSTQDLFLPFFSNVTWFHAIHVSGTNGTKRFDNPVLPFNDGVYFASTEKSNIIRGWIFGTTLDSKTQSLLIVNNATNVVIKVCEFQFCNDPFLGVYYHKNNKSWMESEFRVYSSANNCTFEYVSQPFLMDLEGKQGNFKNLREFVFKNIDGYFKIYSKHTPINLVRDLPQGFSALEPLVDLPIGINITRFQTLLALHRSYLTPGDSSSGWTAGAAAYYVGYLQPRTFLLKYNENGTITDAVDCALDPLSETKCTLKSFTVEKGIYQTSNFRVQPTESIVRFPNITNLCPFGEVFNATRFASVYAWNRKRISNCVADYSVLYNSASFSTFKCYGVSPTKLNDLCFTNVYADSFVIRGDEVRQIAPGQTGKIADYNYKLPDDFTGCVIAWNSNNLDSKVGGNYNYLYRLFRKSNLKPFERDISTEIYQAGSTPCNGVEGFNCYFPLQSYGFQPTNGVGYQPYRVVVLSFELLHAPATVCGPKKSTNLVKNKCVNFNFNGLTGTGVLTESNKKFLPFQQFGRDIADTTDAVRDPQTLEILDITPCSFGGVSVITPGTNTSNQVAVLYQDVNCTEVPVAIHADQLTPTWRVYSTGSNVFQTRAGCLIGAEHVNNSYECDIPIGAGICASYQTQTNSPRAAASVASQSIIAYTMSLGAENSVAYSNNSIAIPTNFTISVTTEILPVSMTKTSVDCTMYICGDSTECSNLLLQYGSFCTQLNRALTGIAVEQDKNTQEVFAQVKQIYKTPPIKDFGGFNFSQILPDPSKPSKRSFIEDLLFNKVTLADAGFIKQYGDCLGDIAARDLICAQKFNGLTVLPPLLTDEMIAQYTSALLAGTITSGWTFGAGAALQIPFAMQMAYRFNGIGVTQNVLYENQKLIANQFNSAIGKIQDSLSSTASALGKLQDVVNQNAQALNTLVKQLSSNFGAISSVLNDILSRLDPPEAEVQIDRLITGRLQSLQTYVTQQLIRAAEIRASANLAATKMSECVLGQSKRVDFCGKGYHLMSFPQSAPHGVVFLHVTYVPAQEKNFTTAPAICHDGKAHFPREGVFVSNGTHWFVTQRNFYEPQIITTDNTFVSGNCDVVIGIVNNTVYDPLQPELDSFKEELDKYFKNHTSPDVDLGDISGINASVVNIQKEIDRLNEVAKNLNESLIDLQELGKYEQYIKWPWYIWLGFIAGLIAIVMVTIMLCCMTSCCSCLKGCCSCGSCCKFDEDDSEPVLKGVKLHYT

SEQ ID NO: 3 - protein, 1256 aa, synthetic construct
MRTLGTCLVTLAGLLLTAAGVNLTTRTQLPPAYTNSFTRGVYYPDKVFRSSVLHSTQDLFLPFFSNVTWFHAIHVSGTNGTKRFDNPVLPFNDGVYFASTEKSNIIRGWIFGTTLDSKTQSLLIVNNATNVVIKVCEFQFCNDPFLGVYYHKNNKSWMESEFRVYSSANNCTFEYVSQPFLMDLEGKQGNFKNLREFVFKNIDGYFKIYSKHTPINLVRDLPQGFSALEPLVDLPIGINITRFQTLLALHRSYLTPGDSSSGWTAGAAAYYVGYLQPRTFLLKYNENGTITDAVDCALDPLSETKCTLKSFTVEKGIYQTSNFRVQPTESIVRFPNITNLCPFGEVFNATRFASVYAWNRKRISNCVADYSVLYNSASFSTFKCYGVSPTKLNDLCFTNVYADSFVIRGDEVRQIAPGQTGKIADYNYKLPDDFTGCVIAWNSNNLDSKVGGNYNYLYRLFRKSNLKPFERDISTEIYQAGSTPCNGVEGFNCYFPLQSYGFQPTNGVGYQPYRVVVLSFELLHAPATVCGPKKSTNLVKNKCVNFNFNGLTGTGVLTESNKKFLPFQQFGRDIADTTDAVRDPQTLEILDITPCSFGGVSVITPGTNTSNQVAVLYQDVNCTEVPVAIHADQLTPTWRVYSTGSNVFQTRAGCLIGAEHVNNSYECDIPIGAGICASYQTQTNSPRAAASVASQSIIAYTMSLGAENSVAYSNNSIAIPTNFTISVTTEILPVSMTKTSVDCTMYICGDSTECSNLLLQYGSFCTQLNRALTGIAVEQDKNTQEVFAQVKQIYKTPPIKDFGGFNFSQILPDPSKPSKRSFIEDLLFNKVTLADAGFIKQYGDCLGDIAARDLICAQKFNGLTVLPPLLTDEMIAQYTSALLAGTITSGWTFGAGAALQIPFAMQMAYRFNGIGVTQNVLYENQKLIANQFNSAIGKIQDSLSSTASALGKLQDVVNQNAQALNTLVKQLSSNFGAISSVLNDILSRLDPPEAEVQIDRLITGRLQSLQTYVTQQLIRAAEIRASANLAATKMSECVLGQSKRVDFCGKGYHLMSFPQSAPHGVVFLHVTYVPAQEKNFTTAPAICHDGKAHFPREGVFVSNGTHWFVTQRNFYEPQIITTDNTFVSGNCDVVIGIVNNTVYDPLQPELDSFKEELDKYFKNHTSPDVDLGDISGINASVVNIQKEIDRLNEVAKNLNESLIDLQELGKYEQYIKWPGGGSGYIPEAPRDGQAYVRKDGEWVLLSTFLGHHHHHH

SEQ ID NO: 4 - protein, 917 aa, synthetic construct
MFVFLVLLPLVSSQCVNLTTRTQLPPAYTNSFTRGVYYPDKVFRSSVLHSTQDLFLPFFSNVTWFHAIHVSGTNGTKRFDNPVLPFNDGVYFASTEKSNIIRGWIFGTTLDSKTQSLLIVNNATNVVIKVCEFQFCNDPFLGVYYHKNNKSWMESEFRVYSSANNCTFEYVSQPFLMDLEGKQGNFKNLREFVFKNIDGYFKIYSKHTPINLVRDLPQGFSALEPLVDLPIGINITRFQTLLALHRSYLTPGDSSSGWTAGAAAYYVGYLQPRTFLLKYNENGTITDAVDCALDPLSETKCTLKSFTVEKGIYQTSNFRVQPTESIVRFPNITNLCPFGEVFNATRFASVYAWNRKRISNCVADYSVLYNSASFSTFKCYGVSPTKLNDLCFTNVYADSFVIRGDEVRQIAPGQTGKIADYNYKLPDDFTGCVIAWNSNNLDSKVGGNYNYLYRLFRKSNLKPFERDISTEIYQAGSTPCNGVEGFNCYFPLQSYGFQPTNGVGYQPYRVVVLSFELLHAPATVCGPKKSTNLVKNKCVNFNFNGLTGTGVLTESNKKFLPFQQFGRDIADTTDAVRDPQTLEILDITPCSFGGVSVITPGTNTSNQVAVLYQDVNCTEVPVAIHADQLTPTWRVYSTGSNVFQTRAGCLIGAEHVNNSYECDIPIGAGICASYQTQTNSPRRAREPKSCDKTHTCPPCPAPELLGGPSVFLFPPKPKDTLMISRTPEVTCVVVDVSHEDPEVKFNWYVDGVEVHNAKTKPREEQYNSTYRVVSVLTVLHQDWLNGKEYKCKVSNKALPAPIEKTISKAKGQPREPQVYTLPPSRDELTKNQVSLTCLVKGFYPSDIAVEWESNGQPENNYKTTPPVLDSDGSFFLYSKLTVDKSRWQQGNVFSCSVMHEALHNHYTQKSLSLSPGK

SEQ ID NO: 5 - DNA, 10155 bp, synthetic construct
  source 1..10155: mol_type = other DNA
  misc_feature 9991: note = betweeb 9991 and 9992, deleted region of 894 bp
accacaggtgggtgctttggaaacttgtcggtcgccgtgctcctgtgagcttgcgtccctccccggtttcctttgcgctcccgccttccggacctgctctcgcctatcttctttggctgtcggtgcgattcgtcaggcagcggccttgtcgaatctcgaccccaccactcgccggacccgccgacgtcccctctggagcccgccgaaacccgccgcgtctgttgaaatggccagccgcccagccgcatcctctcccgtcgaagcgcgggccccggttgggggacaggaggccggcggccccagcgcagccacccagggggaggccgccggggcccctctcgcccacggccaccacgtgtactgccagcgagtcaatggcgtgatggtgctttccaacaagacgcccgggtccgcgtcctaccgcatcagcgatagcaactttgtccaatgtggttccaactgcaccatgatcatagacggagacgtggtgcgcgggcgcccccaggacccgggggccgcggcatcccccgctcccttcgttgcggtgacaaacatcggagccggcagcgacggcgggaccgccgtcgtggcattcgggggaaccccacgtcgctcggcggggacgtctaccggtacccagacgaccgacgtccccaccgaggcccttgggggcccccctcctcctccccgcttcaccctgggtggcggctgttgttcctgtcgcgacacacggcgccgctctgcggtattcgggggggagggggatcccgtcggccccgcggagttcgtctcggacgaccggtcgtccgattccgactcggatgactcggaggacaccgactcggagacgctgtcacacgcctcctcggacgtgtccggcggggccacgtacgacgacgcccttgactccgattcgtcatcggatgactccctgcagatagatggccccgtgtgtcgcccgtggagcaatgacaccgcgcccctggatgtttgccccgggacccccggcccgggcgccgacgccggtggtccctcagcggtagacccacacgcaccgacgccaggggccggcgctggtcttgcggccgatcccgccgtggcccgggacgacgcggaggggctttcggacccccggccacgtctgggaacgggcacggcctaccccgtccccctggaactcacgcccgagaacgcggaggccgtggcgcgctttctgggagatgccgtgaaccgcgaacccgcgctcatgctggagtacttttgccggtgcgcccgcgaggaaaccaagcgtgtcccccccaggacattctgcagcccccctcgcctcacggaggacgactttgggcttctcaactacgcgctcgtggagatgcagcgcctgtgtctggacgttcctccggtcccgccgaacgcatacatgccctattatctcagggagtatgtgacgcggctggtcaacgggttcaagccgctggtgagccggtccgctcgcctttaccgcatcctgggggttctggtgcacctgcggatccggacccgggaggctagagcggccgcatcgaatataacttcgtataatgtatgctatacgaagttatccatggttgatcccgtcgttttacaacgtcgtgactgggaaaaccctggcgttacccaacttaatcgccttgcagcacatccccctttcgccagctggcgtaatagcgaagaggcccgcaccgatcgcccttcccaacagttgcgcagcctgaatggcgaatggcgctttgcctggtttccggcaccagaagcggtgccggaaagctggctggagtgcgatcttcctgaggccgatactgtcgtcgtcccctcaaactggcagatgcacggttacgatgcgcccatctacaccaacgtgacctatcccattacggtcaatccgccgtttgttcccacggagaatccgacgggttgttactcgctcacatttaatgttgatgaaagctggctacaggaaggccagacgcgaattatttttgatggcgttaactcggcgtttcatctgtggtgcaacgggcgctgggtcggttacggccaggacagtcgtttgccgtctgaatttgacctgagcgcatttttacgcgccggagaaaaccgcctcgcggtgatggtgctgcgctggagtgacggcagttatctggaagatcaggatatgtggcggatgagcggcattttccgtgacgtctcgttgctgcataaaccgactacacaaatcagcgatttccatgttgccactcgctttaatgatgatttcagccgcgctgtactggaggctgaagttcagatgtgcggcgagttgcgtgactacctacgggtaacagtttctttatggcagggtgaaacgcaggtcgccagcggcaccgcgcctttcggcggtgaaattatcgatgagcgtggtggttatgccgatcgcgtcacactacgtctgaacgtcgaaaacccgaaactgtggagcgccgaaatcccgaatctctatcgtgcggtggttgaactgcacaccgccgacggcacgctgattgaagcagaagcctgcgatgtcggtttccgcgaggtgcggattgaaaatggtctgctgctgctgaacggcaagccgttgctgattcgaggcgttaaccgtcacgagcatcatcctctgcatggtcaggtcatggatgagcagacgatggtgcaggatatcctgctgatgaagcagaacaactttaacgccgtgcgctgttcgcattatccgaaccatccgctgtggtacacgctgtgcgaccgctacggcctgtatgtggtggatgaagccaatattgaaacccacggcatggtgccaatgaatcgtctgaccgatgatccgcgctggctaccggcgatgagcgaacgcgtaacgcgaatggtgcagcgcgatcgtaatcacccgagtgtgatcatctggtcgctggggaatgaatcaggccacggcgctaatcacgacgcgctgtatcgctggatcaaatctgtcgatccttcccgcccggtgcagtatgaaggcggcggagccgacaccacggccaccgatattatttgcccgatgtacgcgcgcgtggatgaagaccagcccttcccggctgtgccgaaatggtccatcaaaaaatggctttcgctacctggagagacgcgcccgctgatcctttgcgaatacgcccacgcgatgggtaacagtcttggcggtttcgctaaatactggcaggcgtttcgtcagtatccccgtttacagggcggcttcgtctgggactgggtggatcagtcgctgattaaatatgatgaaaacggcaacccgtggtcggcttacggcggtgattttggcgatacgccgaacgatcgccagttctgtatgaacggtctggtctttgccgaccgcacgccgcatccagcgctgacggaagcaaaacaccagcagcagtttttccagttccgtttatccgggcaaaccatcgaagtgaccagcgaatacctgttccgtcatagcgataacgagctcctgcactggatggtggcgctggatggtaagccgctggcaagcggtgaagtgcctctggatgtcgctccacaaggtaaacagttgattgaactgcctgaactaccgcagccggagagcgccgggcaactctggctcacagtacgcgtagtgcaaccgaacgcgaccgcatggtcagaagccgggcacatcagcgcctggcagcagtggcgtctggcggaaaacctcagtgtgacgctccccgccgcgtcccacgccatcccgcatctgaccaccagcgaaatggatttttgcatcgagctgggtaataagcgttggcaatttaaccgccagtcaggctctctttcacagatgtggattggcgataaaaaccaactgctgacgccgctgcgcgatcagttcacccgtgcaccgctggataacgacattggcgtaagtgaagcgacccgcattgaccctaacgcctgggtcgaacgctggaaggcggcgggccattaccaggccgaagcagcgttgttgcagtgcacggcagatacacttgctgatgcggtgctgattacgaccgctcacgcgtggcagcatcaggggaaaaccttatttatcagccggaaaacctaccggattgatggtagtggtcaaatggcgattaccgttgatgttgaagtggcgagcgatacaccgcatccggcgcggattggcctgaactgccagctggcgcaggtagcagagcgggtaaactggctcggattagggccgcaagaaaactatcccgaccgccttactgccgcctgttttgaccgctgggatctgccattgtcagacatgtataccccgtacgtcttcccgagcgaaaacggtctgcgctgcgggacgcgcgaattgaattatggcccacaccagtggcgcggcgacttccagttcaacatcagccgctacagtcaacagcaactgatggaaaccagccatcgccatctgctgcacgcggaagaaggcacatggctgaatatcgacggtttccatatggggattggtggcgacgactcctggagcccgtcagtatcggcggaattccagctgagcgccggtcgctaccattaccagttggtctggtgtcaaaaaaagggcgaattcggtaagcctatccctaaccctctcctcggtctcgattctacgcgtaccgggtgctacgagatttcgattccaccgccgccttctatgaaaggttgggcttcggaatcgttttccgggacgccggctggatgatcctccagcgcggggatctcatgctggagttcttcgcccaccccaacttgtttattgcagcttataatggttacaaataaagcaatagcatcacaaatttcacaaataaagcatttttttcactgcattctagttgtggtttgtccaaactcatcaatgtatcttatcatgtctgtataccgtcgaggctggttctttccgcctcagaagccatagagcccaccgcatccccagcatgcctgctattgtcttcccaatcctcccccttgctgtcctgccccaccccaccccccagaatagaatgacacctactcagacaatgcgatgcaatttcctcattttattaggaaaggacagtgggagtggcaccttccagggtcaaggaaggcacgggggaggggcaaacaacagatggctggcaactagaaggcacagtcgaggctgatcagcgggtttaaactcaatggtgatggtgatgatgaccggtatgcatattcagatcctcttctgagatgagtttttgttcgaaccgcggaagcggccgctatcatgtgtagtgcagtttcacgcccttcagcacgggctcagaatcgtcctcgtcgaacttgcagcagctgccacagctacaacagcccttcaggcagctacagcagctggtcatgcaacacagcatgattgtgaccatcacgatggcaatcagtccggcgataaagcccagccagatgtaccagggccacttgatgtactgctcgtacttccccagttcttgcaggtcgatcaggctctcgttcagattcttggccacctcgttcagccggtcgatctctttctggatgttcacgacgctggcattgattccgctgatatcgcccaggtccacgtcggggcttgtgtggttcttaaagtacttgtccagttcctctttgaagctgtccagctcgggctgcagagggtcgtacacggtattgttcacaatgccgatcacgacgtcgcagttgccagacacgaaggtgttgtcggtggtgatgatctggggctcgtagaagttccgctgtgtcacgaaccaatgggtgccgttggacacgaacacgccttctctaggaaagtgggctttgccgtcgtggcagatggctggagcggtggtgaaattcttctcttgagcgggcacatatgtcacgtgcagaaacaccacgccgtgaggggcagactgagggaagctcatcaggtggtagcccttgccgcaaaagtccactctcttgctctggcccagcacacactcagacatcttggtggcggccagattggcagaggctctaatctcggcggctctgatcagctgctgggtcacgtatgtctggaggctctgcagtctgcctgtgatcagtctgtcgatctgcacctcggcctcaggagggtccagtctgctcaggatatcgttcagcacagagctgatggcgccgaagttggaggacagctgcttgaccagggtgttcagtgcctgggcattctggttgaccacgtcctgcagctttcccagggcgcttgctgtgctgctcaggctgtcctggatcttgccgatggcgctgttgaactggttggcgatcagcttctggttctcgtacagcacattctgggtcactccgatgccgttgaaccggtaggccatctgcatagcaaaggggatctgcagagcggcgccagctccaaatgtccagccgcttgtgattgtgccggccagcagggcagatgtgtactgggcgatcatctcatcggtcagcagaggaggcagcactgtcagtccgttaaacttctgggcgcaaatcagatccctggcggcaatgtcgcccagacaatcgccatactgcttgatgaagccggcgtcggccagtgtcactttgttgaacagcaggtcctcgatgaagctccgcttgctgggcttgctaggatcgggcagaatctggctgaaattgaagccgccgaagtccttgataggaggggtcttgtagatctgcttcacttgggcgaacacctcttgggtgttcttgtcctgttccacggcgatccctgtcagggctctattcagctgggtgcagaagctgccgtactgcagcagcaggttggagcactcggtggaatcgccgcagatgtacatggtgcagtccacgctggtcttggtcatggacacaggcaggatctctgtggtcacgctgatggtgaagttggtggggatagcgatagagttgttggagtaggccacgctgttctcggcgcccagagacattgtgtaggcaatgatgctctggctggccacagatctggcccgtctggggctgtttgtctgtgtctggtagctggcacagatgccagcgccgatggggatgtcgcactcgtagctattgttcacgtgctcggctccgatcagacagccggctctggtctgaaacacattgctgccggtggagtacacccgccatgtaggtgtcagctgatcggcgtgaatggccacgggcacttcggtacagttcacgtcctggtacagcactgccacctgattgctggtgttggtgccaggggtgatcacagacactccgccgaagctgcaaggggtgatgtccaggatttccagtgtctggggatctctaacggcgtctgtggtatcggcgatatcccggccaaactgctggaatggcaggaacttcttgttgctctctgtcagcacgccggtgccggtcaggccgttgaagttgaagttcacgcatttgttcttcacgagattggtgcttttcttagggccgcacactgtggcaggggcatgcagcagttcgaagctcagcaccaccactctgtagggctgatagcccacgccatttgtgggctgaaagccgtaggactgcagtgggaagtagcagttgaagccttccacgccgttacaaggggtgctgccggcctgatagatctcggtggagatgtcccgctcgaagggcttcagattggacttccggaacagccggtacaggtaattgtagttgccgccgactttggagtccaggttgttgctgttccaggcaatcacacagccggtgaagtcgtcgggcagcttgtagttgtagtcggcgatcttgcctgtctgtccaggggcaatctgccgcacttcatctccccggatcacgaagctgtcggcgtacacgtttgtgaagcacaggtcgttcagcttggtaggggacacgccgtagcacttgaaggtgctgaagctggcggagttgtacagcacggagtagtcggccacgcaattgctgatccgcttccggttccaggcgtacacagaggcgaatctggtggcattgaacacctcgccgaaggggcacagattggtgatattggggaaccgcacgatggattcggtgggctgcacccggaagttgctggtctggtagatgcccttttccacggtgaaggacttcagggtgcactttgtctcgctcagaggatcaagggcacaatccacggcgtcggtgatggtgccgttctcgttgtacttcagcaggaaggttctaggctgcaggtagcccacatagtaagcggcggcaccagctgtccatccgctgctgctatcgccaggtgtcaggtagcttctgtgcagggccagcagtgtctgaaaccgggtgatgttgatgccgatgggcagatccaccaggggttccagagcagagaagccctgaggcagatcccgcacgaggttgataggggtgtgcttgctgtagatcttgaagtagccgtcgatgttcttgaacacgaactcgcgcaggttcttgaagttgccctgcttgccttccaggtccatcaggaaaggctgggacacgtactcgaaggtgcagttgttggcgctgctgtacacccggaactcgctttccatccagctcttgttgttcttgtggtagtagacgcccaggaaggggtcgttgcagaactggaactcgcacactttgatgaccacgttggtggcgttgttcacgatcagcaggctctgggtcttgctgtccagtgtggtgccgaagatccagcctctgatgatgttggacttctcggtgctggcaaagtacaccccgtcgttgaagggcagcacggggttgtcgaatctcttggtgccattggtgccggacacgtggatggcgtggaaccaggtcacgttgctgaagaaaggcaggaacaggtcctgggtagagtgcagcacgctggatctgaacaccttgtcggggtagtacacgcctctggtaaagctgttggtgtaggctggaggcagctgtgttctggtggtcaggttcacacactggctggacaccagaggcagcagcaccagaaacacgaacatggtggcggatccggatccgagctcggtaccaagcttaactagccagcttgggtctccctatagtgagtcgtattaatttcgataagccagtaagcagtgggttctctagttagccagagagctctgcttatatagacctcccaccgtacacgcctaccgcccatttgcgtcaatggggcggagttgttacgacattttggaaagtcccgttgattttggtgccaaaacaaactcccattgacgtcaatggggtggagacttggaaatccccgtgagtcaaaccgctatccacgcccattgatgtactgccaaaaccgcatcaccatggtaatagcgatgactaatacgtagatgtactgccaagtaggaaagtcccataaggtcatgtactgggcataatgccaggcgggccatttaccgtcattgacgtcaatagggggcgtacttggcatatgatacacttgatgtactgccaagtgggcagtttaccgtaaatactccacccattgacgtcaatggaaagtccctattggcgttactatgggaacatacgtcattattgacgtcaatgggcgggggtcgttgggcggtcagccaggcgggccatttaccgtaagttatgtaacgcggaactccatatatgggctatgaactaatgaccccgtaattgattactattaataactagtcaataatcaatgtcaacgcgtatatctggcccgtacatcgcctgtcgacatttaaatgctagcggtacccttaagcctgcaggactagtactgatccgaagttcctatactttctagagaataggaacttcctcgaggtcatggggttcggcgagcagatacccatccaggagctggcctatggcattgtgcgcagtgcggccacgaccgggagccccttcgtcatgttcaaagacgcggtgaaccgccactacatctacgacacccagggggcggccatcgccggctccaacctc

SEQ ID NO: 6 - DNA, 1450 bp, synthetic construct
  source 1..1450: mol_type = other DNA
agcgagttagacaggcaagcactactcgcctctgcacgcacatgcttgcctgtcaaactctaccaccccggcacgctctctgtctccatggcccgccgccgccgccatcgcggcccccgccgcccccggccgcccgggcccacgggcgccgtcccaaccgcacagtcccaggtaacctccacgcccaactcggaacccgcggtcaggagcgcgcccgcggccgccccgccgccgccccccgccagtgggcccccgccttcttgttcgctgctgctgcgccagtggctccacgttcccgagtccgcgtccgacgacgacgatgacgacgactggccggacagccccccgcccgagccggcgccagaggcccggcccaccgccgccgccccccgcccccggtccccaccgcccggcgcgggcccggggggcggggctaacccctcccaccccccctcacgccccttccgccttccgccgcgcctcgccctccgcctgcgcgtcaccgcagagcacctggcgcgcctgcgcctgcgacgcgcgggcggggagggggcgccggagccccccgcgacccccgcgacccccgcgacccccgcgacccccgcgacccccgcgcgggtgcgcttctcgccccacgtccgggtgcgccacctggtggtctgggcctcggccgcccgcctggcgcgccgcggctcgtgggcccgcgagcgggccgaccgggctcggttccggcgccgggtggcggaggccgaggcggtcatcgggccgtgcctggggcccgaggcccgtgcccgggccctggcccgcggagccggcccggcgaactcggtctaacgttacacccgaggcggcctgggtcttccgcggagctcccgggagctccgcaccaagccgctctccggagagacgatggcaggagccgcgcatatatacgctgggagccggcccgcccccgaggcgggcccgccctcggagggcgggactggccaatcggcggccgccagcgcggcggggcccggccaaccagcgtccgccgagtcttcggggcccggcccactgggcgggagttaccgcccagtgggccgggccgcccacttcccggtatggtaattaaaaacttacaagaggccttgttccgcttcccggtatggtaattagaaactcattaatgggcggccccggccgcccttcccgcttccggcaattcccgcggcccttaatgggcaaccccggtattccccgcctcccgcgccgcgcgtaaccactcccctggggttccgggttatgctaattgcttttttggcggaacacacggcccctcgcgcattggcccgcgggtcgctcaatgaacccgcattggtcccctggggttccgggtatggtaatgagtttcttcgggaaggcgggaagccccggggcaccgacgcaggccaagcccctgttgcgtcgg

SEQ ID NO: 7 - DNA, 707 bp, synthetic construct
  source 1..707: mol_type = other DNA
attatcaccccgttgcgggggtccggagatcatgcgcgggtgtcctcgaggtgcgtgaacacctctggggtgcatgccggcggacggcacgccttttaagtaaacatctgggtcgcccggcccaactggggccgggggttgggtctggctcatctcgagagccacgggggggaaccaccctccgcccagagactcgggtgatggtcgtacccgggactcaacgggttaccggattacggggactgtcggtcacggtcccgccggttcttcgatgtgccacacccaaggatgcgttgggggcgatttcgggcagcagcccgggagagcgcagcaggggacgctccgggtcgtgcacggcggttctggccgcctcccggtcctcacgcccccttttattgatctcatcgcgtacgtcggcgtacgtcctgggcccaacccgcatggtgtccaggaaggtgtccgccatttccagggcccacgacatgctcccccccgacgagcaggaagcggtccacgcaacggtcgccgccggtcgcctcgacgaggacgttcctcctgcgggaaggcacgaacgcgggtgagccccctcctccgcccccgcgtcccccctcctccgcccccgcgtcccccctcctccgcccccgcgtcccccctcctccgcccccgcgtcccccctcctccgcccccgcgtcccccctcctccgccc